European Patent Application EP 4 722 342 A1, published April 8, 2026. Title: A cell line for culturing african swine fever virus and vaccine using the same. Applicant: Choong Ang Vaccine Lab. Application KR. The sequence listing filed with the application follows.

SEQUENCE LISTING (2 sequences)

SEQ ID NO: 1 - DNA, 25 bp, synthetic construct
  source 1..25: mol_type = other DNA
ctgctcatggtatcaatcttatcga

SEQ ID NO: 2 - DNA, 21 bp, synthetic construct
  source 1..21: mol_type = other DNA
gataccacaagatcaggccgt